European Patent Specification EP 3 066 200 B1, published December 4, 2024. Title: Compositions and Methods for Controlling Arthropod Parasite and Pest Infestations. Applicant: Monsanto Technology LLC Beeologics Inc The United States of America,as represented by the Secretary of Agriculture Inberg, Alex Kapoor, Mahak Evans, Jay. The sequence listing filed with the application follows.

SEQUENCE LISTING (89 sequences)

SEQ ID NO: 1 - DNA, 450 bp, Varroa destructor
atggctgatcagctaactgaggaacagatcgccgagttcaaagaggcgtttagcctgtttgacaaggacggagatggcacgatcacgacaaaggagctcggtacggtaatgcgatctctcggccagaaccccactgaggctgaactgcaggacatgatcaacgaggtcgacgccgacggctccggaacgatagatttccctgagttcctcacaatgatggcaagaaagatgaaggacaccgactcggaggaggagatccgagaggcgttccgcgtattcgacaaggatggcaacggtttcatttcggcggccgagctcaggcacgttatgaccaaccttggcgagaagcttacggacgaggaggtagatgagatgattcgggaggcagatattgacggtgatggtcaggtcaactacgaggagttcgtcaccatgatgacgtccaagtaa

SEQ ID NO: 2 - DNA, 450 bp, Varroa destructor
atggcggatcagctgaccgaggagcaaatcgccgaattcaaggaggctttcagcctgttcgataaagacggtgatggcacaattacgaccaaggaactagggaccgtcatgcggtccctcggccagaaccctactgaggctgagcttcaagacatgatcaacgaggtcgacgctgacggtaacggcactattgactttccagagtttctcacgatgatggcgcgtaaaatgaaggacaccgactccgaggaggagatccgggaagcttttagggtttttgataaagacggaaatggcttcatttcggctgcagagctgaggcacgtaatgaccaaccttggcgaaaagctcacggacgaggaagtggacgagatgatccgcgaggcggatatcgacggcgacggacaggtcaactacgaggagttcgtcacgatgatgacatcaaaatga

SEQ ID NO: 3 - RNA, 373 nt, Varroa destructor
acagaucgccgaguucaaagaggcguuuagccuguuugacaaggacggagauggcacgaucacgacaaaggagcucgguacgguaaugcgaucucucggccagaaccccacugaggcugaacugcaggacaugaucaacgaggucgacgccgacggcuccggaacgauagauuucccugaguuccucacaaugauggcaagaaagaugaaggacaccgacucggaggaggagauccgagaggcguuccgcguauucgacaaggauggcaacgguuucauuucggcggccgagcucaggcacguuaugaccaaccuuggcgagaagcuuacggacgaggagguagaugagaugauucgggaggcagauauugac

SEQ ID NO: 4 - RNA, 186 nt, Varroa destructor
acaaugauggcaagaaagaugaaggacaccgacucggaggaggagauccgagaggcguuccgcguauucgacaaggauggcaacgguuucauuucggcggccgagcucaggcacguuaugaccaaccuuggcgagaagcuuacggacgaggagguagaugagaugauucgggaggcagauauugac

SEQ ID NO: 5 - RNA, 274 nt, Unkown
auacuuacuggugcuaauuuuuaucgaggaugcccaacuccccccacuuuaaaacugcgaucauacuaacgaacucccgaaggagugaaaggugucuauguugagcuuaauaaccuaccuugcgagcaaagaaggacuaguugacccugggcacccuauauuguuauguuguuucgaacugaguuggcacccaugcugcacaugcaacaaacaugucggccuucgugucuauccuagaaaaguaccugugaacuuggcugucuacaucaucauc

SEQ ID NO: 6 - DNA, 432 bp, Varroa destructor
ctgccggaggaacaggtggctgaatttaaagaggcctttcttttgtttgacaaggacgccgatggaatgattacggccgccgaactaggcgtcgtcatgcgatcgcttggccagcgacctacggagcaagagctcaagaaaatggttaccatggttgaccaggacggcaatggtacaatcgagttcaacgagtttttgatgatgatgtctcgcaagatgaaggaggcagactcggaggaagaactccgggaggcgttccgtgtgttcgatcgagacggtgacggattcatctcgcgggacgagctcagtgtcgtcatgaacaacctcggcgagaaattaagtgacgatgatgttgaggatatgattcgagaggccgatctggacggcgatggcaagattaactaccaagagtttgtgctcattatcacctcc

SEQ ID NO: 7 - DNA, 480 bp, Ixodes scapularis
atggctgatcagcttacagaagaacagattgcagttcaaggaggcgttcttcgctgttcgacaaggacggaggatggcaccatcacgaccaaggagctgggcacggtcatgcgctcgctcggccagaacccgacggaggcggagctgcaggacatgatcaacgaggtggacgcagacggcaacggaacgatcgacttccccgagttccttacgatgatggcgcgcaagatgaaggacacggactctgaggaggagatccgggaggcgttccgggtgttcgacaaggacggcaacggcttcatctctgcggcggagctgcgccacgtcatgaccaacctgggcgagaagctgacggacgaggaggtggacgagatgatccgggaggcggacatcgacggggacgggcaggtcaactacgaaggtgggcacgctttccctcccttggttatcctcctgctatgctttctgcagttgctgtga

SEQ ID NO: 8 - DNA, 450 bp, Aedes aegypti
atggccgatcaacttacagaagagcagattgccgaattcaaagaagcgttttcgctgttcgacaaagacggtgacggcacaatcacaaccaaggaactgggaaccgtgatgcgatcgttaggccagaaccccacagaagcagaactgcaagatatgataaacgaagtcgacgcggacggcaacggcacgatcgatttccccgaattcctgaccatgatggctcgcaaaatgaaggacaccgatagcgaagaggaaatccgggaggcgttccgagtcttcgacaaggacggcaacggcttcatctcggcagctgagctgcgtcatgtcatgaccaatctcggcgagaagctaacggacgaggaggtggatgagatgatccgcgaagccgacatagatggcgatggccaagttaattatgaagaattcgtaacaatgatgacatcgaagtga

SEQ ID NO: 9 - DNA, 450 bp, Culex quinquefasciatus
atggccgatcaacttacagaggaacagatcgccgagttcaaagaagcgttctcgctgttcgacaaagacggtgacggcacgatcacgaccaaggagctgggcaccgtgatgcgatcgttaggccagaaccccacagaagcagagctgcaagacatgataaacgaggtcgatgcggacggcaacggcacgatcgacttccccgagtttctcaccatgatggctcgcaaaatgaaggacaccgatagcgaagaggaaatccgggaggcgttccgagtcttcgacaaggacggcaacggcttcatctcggcggccgagctgcgccacgtcatgaccaatctcggcgagaagctcacggacgaggaggtggatgagatgatccgcgaggccgacattgacggcgatggccaagttaattatgaagaattcgtaacaatgatgacatcgaagtga

SEQ ID NO: 10 - DNA, 450 bp, Acyrthosiphon pisum
atggctgatcaactaacagaagaacagattgccgaattcaaagaggcgttttcgctattcgacaaggacggagatggtaccatcaccaccaaagaacttggaaccgtcatgaggtctttaggccaaaatccgactgaagctgaactccaagatatgattaacgaggtcgatgctgatggcaacggcacgatagatttcccagagttcttgactatgatggcccgcaaaatgaaggataccgatagtgaggaagaaatcagagaggctttccgtgtatttgataaggatggaaacggctttattagtgcagctgagctgcgtcatgtgatgactaaccttggagaaaagctcaccgatgaagaggttgatgaaatgatcagggaagctgacattgatggtgatggtcaagtcaactatgaagagttcgtgaccatgatgacttctaagtga

SEQ ID NO: 11 - DNA, 441 bp, Harpegnathos saltator
caactcacagaggaacagatcgcagagtttaaggaagccttctcgctattcgacaaagatggcgatggcactataacgactaaagaattgggtacagtcatgcgatccctgggtcaaaatcccacagaggccgagttacaagacatgattaatgaagtagacgcagatggtaacggtacaatcgactttccggagttcttgaccatgatggcacgcaaaatgaaggatacggacagcgaggaggagatcagggaggccttcagagtgttcgataaggatggaaatggtttcatatccgcagcggaactcagacatgttatgacaaatctgggcgagaaactgaccgatgaggaagtagatgaaatgatacgggaggcagatatcgacggcgatggccaagtgaattatgaagaatttgtgacgatgatgacatcaaagtga

SEQ ID NO: 12 - DNA, 459 bp, Pediculus humanus corporis
atggtttctttttttttgcgagctgatcagttgaccgaagaacaaattgccgaattcaaggaagcattttccttattcgacaaagatggcgatggtaccataacaactaaggaattgggtacggttatgagatcactcggtcagaatcccacagaagcagaattacaagatatgattaatgaagtggatgcagatggtaatggtaccatcgattttcccgagttcctcaccatgatggctagaaaaatgaaggatacagacagcgaagaagaaattagagaagcattcagagttttcgataaggatggtaatggttttatatcggcagccgagctaaggcacgtcatgacgaacctgggtgaaaaattaacagacgaagaagtggatgaaatgattcgagaggctgatatcgacggagatggacaagtgaattacgaagaatttgtggaaaacttgtga

SEQ ID NO: 13 - DNA, 459 bp, Anopheles gambiae
atggccgatcaacttacggaagaacagatcgctgaattcaaagaagcgttctcgctgttcgacaaggacggcgatggcacaatcaccaccaaggaattaggcaccgtgatgcgatcgctaggccagaaccccacagaagctgaattgcaagacatgatcaacgaagtcgacgcggacggtaacggcacgatcgatttccccgagtttctaacaatgatggctcgtaaaatgaaggacacggacagtgaagaggaaatccgggaggcattccgagtcttcgacaaggacggcaacggttttatctctgcagctgagctgcgccacgtcatgactaatctgggcgagaagctaacagacgaggaggtcgacgagatgatccgtgaagccgatatagatggcgatggccaggttaattatgaaggtaagagttgcctttcgcgcccacaccaagcattgttt

SEQ ID NO: 14 - DNA, 501 bp, Solenopsis invicta
atgatcggcacgataacgacgagaaattccattatttcagaattcaaagaggcatttatgcttttcgacaaggacgaagatggcacgattacgatggcggaattaggggttgtcatgcggtctctcggtcaaagaccgtcggagacggaactgcgcgatatggtgaatgaggtagatcaagatggaaatggtaccatcgagtttaacgaatttctgcagatgatgtcgaagaagatgaaaagcgccgacggagaggacgaacttcgcgaggcgttccgagtgttcgataagaacaacgatggcttaatatcttcgaaagagttgcgacacgtaatgacgaatcttggtgaaaagctctctgaggaggaggtcgatgatatgattaaggaggcggatctagatggcgacggaatggtcaactacgaaggtaacattttgttttgcctagatgtttattctataatagatttagaatttattctaagcgatatagatgaattg

SEQ ID NO: 15 - RNA, 364 nt, Ixodes scapularis
aguucaaggaggcguucuucgcuguucgacaaggacggaggauggcaccaucacgaccaaggagcugggcacggucaugcgcucgcucggccagaacccgacggaggcggagcugcaggacaugaucaacgagguggacgcagacggcaacggaacgaucgacuuccccgaguuccuuacgaugauggcgcgcaagaugaaggacacggacucugaggaggagauccgggaggcguuccggguguucgacaaggacggcaacggcuucaucucugcggcggagcugcgccacgucaugaccaaccugggcgagaagcugacggacgaggagguggacgagaugauccgggaggcggacaucgac

SEQ ID NO: 16 - RNA, 372 nt, Aedes aegypti
gcagauugccgaauucaaagaagcguuuucgcuguucgacaaagacggugacggcacaaucacaaccaaggaacugggaaccgugaugcgaucguuaggccagaaccccacagaagcagaacugcaagauaugauaaacgaagucgacgcggacggcaacggcacgaucgauuuccccgaauuccugaccaugauggcucgcaaaaugaaggacaccgauagcgaagaggaaauccgggaggcguuccgagucuucgacaaggacggcaacggcuucaucucggcagcugagcugcgucaugucaugaccaaucucggcgagaagcuaacggacgaggagguggaugagaugauccgcgaagccgacauaga

SEQ ID NO: 17 - RNA, 373 nt, Culex quinquefasciatus
acagaucgccgaguucaaagaagcguucucgcuguucgacaaagacggugacggcacgaucacgaccaaggagcugggcaccgugaugcgaucguuaggccagaaccccacagaagcagagcugcaagacaugauaaacgaggucgaugcggacggcaacggcacgaucgacuuccccgaguuucucaccaugauggcucgcaaaaugaaggacaccgauagcgaagaggaaauccgggaggcguuccgagucuucgacaaggacggcaacggcuucaucucggcggccgagcugcgccacgucaugaccaaucucggcgagaagcucacggacgaggagguggaugagaugauccgcgaggccgacauugac

SEQ ID NO: 18 - RNA, 372 nt, Acyrthosiphon pisum
acagauugccgaauucaaagaggcguuuucgcuauucgacaaggacggagaugguaccaucaccaccaaagaacuuggaaccgucaugaggucuuuaggccaaaauccgacugaagcugaacuccaagauaugauuaacgaggucgaugcugauggcaacggcacgauagauuucccagaguucuugacuaugauggcccgcaaaaugaaggauaccgauagugaggaagaaaucagagaggcuuuccguguauuugauaaggauggaaacggcuuuauuagugcagcugagcugcgucaugugaugacuaaccuuggagaaaagcucaccgaugaagagguugaugaaaugaucagggaagcugacauuga

SEQ ID NO: 19 - RNA, 373 nt, Harpegnathos saltator
acagaucgcagaguuuaaggaagccuucucgcuauucgacaaagauggcgauggcacuauaacgacuaaagaauuggguacagucaugcgaucccugggucaaaaucccacagaggccgaguuacaagacaugauuaaugaaguagacgcagaugguaacgguacaaucgacuuuccggaguucuugaccaugauggcacgcaaaaugaaggauacggacagcgaggaggagaucagggaggccuucagaguguucgauaaggauggaaaugguuucauauccgcagcggaacucagacauguuaugacaaaucugggcgagaaacugaccgaugaggaaguagaugaaaugauacgggaggcagauaucgac

SEQ ID NO: 20 - RNA, 373 nt, Pediculus humanus corporis
acaaauugccgaauucaaggaagcauuuuccuuauucgacaaagauggcgaugguaccauaacaacuaaggaauuggguacgguuaugagaucacucggucagaaucccacagaagcagaauuacaagauaugauuaaugaaguggaugcagaugguaaugguaccaucgauuuucccgaguuccucaccaugauggcuagaaaaaugaaggauacagacagcgaagaagaaauuagagaagcauucagaguuuucgauaaggaugguaaugguuuuauaucggcagccgagcuaaggcacgucaugacgaaccugggugaaaaauuaacagacgaagaaguggaugaaaugauucgagaggcugauaucgac

SEQ ID NO: 21 - RNA, 372 nt, Anopheles gambiae
acagaucgcugaauucaaagaagcguucucgcuguucgacaaggacggcgauggcacaaucaccaccaaggaauuaggcaccgugaugcgaucgcuaggccagaaccccacagaagcugaauugcaagacaugaucaacgaagucgacgcggacgguaacggcacgaucgauuuccccgaguuucuaacaaugauggcucguaaaaugaaggacacggacagugaagaggaaauccgggaggcauuccgagucuucgacaaggacggcaacgguuuuaucucugcagcugagcugcgccacgucaugacuaaucugggcgagaagcuaacagacgaggaggucgacgagaugauccgugaagccgauauaga

SEQ ID NO: 22 - RNA, 364 nt, Solenopsis invicta
cagaauucaaagaggcauuuaugcuuuucgacaaggacgaagauggcacgauuacgauggcggaauuagggguugucaugcggucucucggucaaagaccgucggagacggaacugcgcgauauggugaaugagguagaucaagauggaaaugguaccaucgaguuuaacgaauuucugcagaugaugucgaagaagaugaaaagcgccgacggagaggacgaacuucgcgaggcguuccgaguguucgauaagaacaacgauggcuuaauaucuucgaaagaguugcgacacguaaugacgaaucuuggugaaaagcucucugaggaggaggucgaugauaugauuaaggaggcggaucuaga

SEQ ID NO: 23 - RNA, 373 nt, Varroa destructor
acagguggcugaauuuaaagaggccuuucuuuuguuugacaaggacgccgauggaaugauuacggccgccgaacuaggcgucgucaugcgaucgcuuggccagcgaccuacggagcaagagcucaagaaaaugguuaccaugguugaccaggacggcaaugguacaaucgaguucaacgaguuuuugaugaugaugucucgcaagaugaaggaggcagacucggaggaagaacuccgggaggcguuccguguguucgaucgagacggugacggauucaucucgcgggacgagcucagugucgucaugaacaaccucggcgagaaauuaagugacgaugauguugaggauaugauucgagaggccgaucuggac

SEQ ID NO: 24 - DNA, 627 bp, Tetranychus urticae
attcatcagatttaaaattattcaccttgtacctgaattaaaacaatagtattatataagatggctgaccagctaactgaagagcaaattgctgaatttaaggaggccttttcattgtttgataaagatggtgatggtacaattaccaccaaggaattgggaactgttatgagaagtctaggtcaaaatccaacagaagcggaattacaagatatgatcaatgaagttgatgccgatggtaatggtactattgattttcctgaattcttgactatgatggctagaaaaatgaaggatacagactcagaggaggaaatccgtgaagctttccgtgtttttgataaagatggtaatggttttatttctgctgctgaattgagacatgtaatgaccaatttgggtgaaaaattgaccgacgaagaagtagatgaaatgattcgtgaagccgatattgacggtgatggtcaagttaattatgaagaatttgtaacgatgatgacatccaaatgaataaaagcacaaggttaattgttcattttaattagatccaatggatcccatcagtgacagggataaaaattaatcaataaaagatgaaaagcaaaaaatacatggaagctatcatca

SEQ ID NO: 25 - RNA, 372 nt, Tetranychus urticae
caaauugcugaauuuaaggaggccuuuucauuguuugauaaagauggugaugguacaauuaccaccaaggaauugggaacuguuaugagaagucuaggucaaaauccaacagaagcggaauuacaagauaugaucaaugaaguugaugccgaugguaaugguacuauugauuuuccugaauucuugacuaugauggcuagaaaaaugaaggauacagacucagaggaggaaauccgugaagcuuuccguguuuuugauaaagaugguaaugguuuuauuucugcugcugaauugagacauguaaugaccaauuugggugaaaaauugaccgacgaagaaguagaugaaaugauucgugaagccgauauugac

SEQ ID NO: 26 - DNA, 1114 bp, Varroa destructor
  unsure (1)..(1114): unsure at all n locations
  misc_feature (1100)..(1110): n is a, c, g, or t
ggctcgtacaccgagagagaacggtggactccattgctgtcctgagtgcgtttctcgtcggctgtgtcgtattgcgtgtctgtccgtgctttcgtgcacataagttttctttccacattggagatattgtgaatagtatcctttgtgtttagtgcctgaacaatatttgaaatcgtcgaacgtatcaagacataaaaacgagccaaaatggctgatcaacttacggaagaacaaatcgcagaatttaaggaagcattttcactatttgataaagatggagatggtaccatcacaactaaagagttgggtacagttatgcgatcactaggtcaaaatcccacagaagctgagcttcaggatatgattaatgaagttgatgcagatggtaatggcacaatcgattttccggaattcttaactatgatggctcgtaaaatgaaagatactgatagtgaggaagaaattagggaggccttcagagtatttgataaggatggaaatggtttcatatccgcagcagaactcagacatgttatgacaaatcttggcgagaaactcactgatgaagaagttgatgaaatgattcgggaggctgacattgatggtgatggccaagttaattatgaagaattcgtcacaatgatgacatcaaagtgaatgcaacctgtgtaatggaaaaacttgcaacttggagtggtgttgacgtattaagataaatcaagaaacaaagaaaaatataatgttaacaaaaaacgaatcgaccagaaagtgaaaaaaatcttgtatctggacgcaaagatgtctataaaacgcgaaaaattaacgtccaacacgcgttaatcatcattaacgataagtaatacagggcaattgtttaattaaaagagttataccactaaaaatcattatctctaaatacacaaaacttaattacacaacatgaacataaaaatacatattactcgcgcacatacatgaatacaaaaaaatatacagcacacagaaataccatctacataaaagataatttatttccgtattaaaaagtatataattaaaaaatgttagagatatatatatataatatatatatatatatnnnnnnnnnnngtaa

SEQ ID NO: 27 - RNA, 372 nt, Varroa destructor
acaaaucgcagaauuuaaggaagcauuuucacuauuugauaaagauggagaugguaccaucacaacuaaagaguuggguacaguuaugcgaucacuaggucaaaaucccacagaagcugagcuucaggauaugauuaaugaaguugaugcagaugguaauggcacaaucgauuuuccggaauucuuaacuaugauggcucguaaaaugaaagauacugauagugaggaagaaauuagggaggccuucagaguauuugauaaggauggaaaugguuucauauccgcagcagaacucagacauguuaugacaaaucuuggcgagaaacucacugaugaagaaguugaugaaaugauucgggaggcugacauuga

SEQ ID NO: 28 - DNA, 822 bp, Varroa destructor
ttttttttttttttcgaagaaatcgtatcatcgaacatcggatcgaatttcgatccacgacgctcgaattacatgcaacgaagtgaatgtcagaggggggggggcaggggaaaagtatgcgacgaacgtgtacgtccgtcgtccgctggctcgtcgttaattcgttctatctaacacagacacgagaataagtaagatcctagtagcccggggacagcacctcctcctcctcgtcctcctcgtcgtcgtcgatccccggctctccgagcgcgtggacgaattcgtagaaatcgatacggccgtctccgtccacgtccacttccttgatcatatcctcgatctcttcttccgacaagtcctcgccgagacattgcagcactgccctcaaatcggatgcggtgatgtatcctcgattgtgtttatcgaatacccggaacgcatccctcagctcctgctcttcctgatcctgatccgtgggggcggtttcattcgcacctatgttgctcacgatttccacgaactcttcgaagctgacatttccatccccgtcgatgtcgatctcctgcaacatggtgcgcagctcctcggccctcgcgaattgccccaacgagcgcatcaccctcccgagctcctccttcgtgatgctcccgtccccgtccttgtcgaacagtctgaacgcttccctgaattctttcatttgagatttggatatattgctcggtatcttggtggacgactcagaggcggattttttcggcgacgcaggtaaggagaagaggacgttggtcgacaatttgccggcctccgtggacgaggaggccg

SEQ ID NO: 29 - RNA, 300 nt, Varroa destructor
aacguguacguccgucguccgcuggcucgucguuaauucguucuaucuaacacagacacgagaauaaguaagauccuaguagcccggggacagcaccuccuccuccucguccuccucgucgucgucgauccccggcucuccgagcgcguggacgaauucguagaaaucgauacggccgucuccguccacguccacuuccuugaucauauccucgaucucuucuuccgacaaguccucgccgagacauugcagcacugcccucaaaucggaugcggugauguauccucgauuguguuuauc

SEQ ID NO: 30 - DNA, 2577 bp, Varroa destructor
ctgctgctgctgctgctgctgctgctgccgtgttaagaactagacaaaggcaacaaccggaagacatctgttaggccagttgggtgaagggaaataaactcgcaacaaagagctactgttgcaaaagctatctgttctgagtcctagactagactgggatcgactaacaactctgcaggccgtggaccactatcactgaacaacgccgcaggaccgagcgattgagaagttggccgcggctgggacgctctggctcacttgatctgattactacttacaccaggtcaatttaaccaagccgttgaaccactcctacatggaaacacacatctacactctcatccaattgtgtacacgcgaagcaaacgacaacggtattagcagcgacactaacaaaaacgaatctgccagaaaccgagtaacgctgatttctgcagcggcgttcctacgaacttaccacagacccggtcggcacaatagtttgaaggttagcatcggcccgtgaactatagtgaaaggaactgagcgaaatactatagttgttgaacagcaggcttcaaagtaaagaagtgaatattcttatggtgacaacaaattttgtctgtagtggtcaagaccctactcaatgaagtgagaagcgaattcatatgtgctcagttatagcagttgtttgtcgtaatgccgccaatatacgacgtctgtgtgtctcgatactggcgtatctgactgattccgatcggtgtcattgatctgcaaagccaattgttttctttacgtcccggatagagcaaacgatcatggcaacggaaacatttggcctgccggaggaacaggtggctgaatttaaagaggcctttcttttgtttgacaaggacgccgatggaatgattacggccgccgaactaggcgtcgtcatgcgatcgcttggccagcgacctacggagcaagagctcaagaaaatggttaccatggttgaccaggacggcaatggtacaatcgagttcaacgagtttttgatgatgatgtctcgcaagatgaaggaggcagactcggaggaagaactccgggaggcgttccgtgtgttcgatcgagacggtgacggattcatctcgcgggacgagctcagtgtcgtcatgaacaacctcggcgagaaattaagtgacgatgatgttgaggatatgattcgagaggccgatctggacggcgatggcaagattaactaccaagagtttgtgctcattatcacctccgccaagtaggccttggagttgctcgcgcacacacatgctattcctcttgtcctacacgacaaacactatacacgttacaatacggaaaaatgaaataaaagcacagtcacacttattcattcattcacagaggatcactggcgtgtcctcattaatatggctgacaaatactattgatttgtctcgactgagctatcaggcacacgcatattgtctgttccgatacgtgcaataataggtaaagtggtgttagcttgagcaccttacggtttacatttattccgtattaacggtactatgtctcaatagtcatgtcgcagcattagccagctaacattaaatttagttgatttttattttatttttttacacaacaagaattatcttactatttggcaagctgactgcgagtagtaaaattaccctagtaaaaaaaaaaggctttaaaaacgatttaacaaaggtgcgtccatttaaaaaagtatgacacaagctaatgtgttcgatcgcggtcggttgcattcggccagtttgtgagacgcgaaatttaccagcagccgtcaacaacgatggaataattatatattaaatataaataataaaatatctgttacacattctatgtgaataaagttatacatatatatatacatacaacagcaatgatatatatgatgatacgtatactatatagaagtatccactgatataggataatgggaaattctggaaaggagaaaacatattcttctttcataattaatgaattatcatcgagcacctcaagaatttgcttagacatattacaaaaaaaaaattaattcactatatataaataatcgcaattaatcaaaaaaaaaatacggtcatttatggcataccctaggttaataaacttcataaaggtacctatatatatatcttttttactgtctctttaatcgtcattatacatagtgacgattaaagagagagagtaaaaaagaggtcaaaataaaagacttgaagtcgattgaggttaatttttattctaggttatatgtgttttagcggatttatagtgtgctcgttgtaaaagttgacgtaaggagttgaaacgcggagagcagtataacagtaaaatggagaggaagtttagaagttgggaaataaatgatttgctactaattggaaattacaaaaatgaccatttaaagaacttatcattagaattttaatatctgccacactgaaccgttttgtcattatttcgaccatagcgattttcacacagttgtctcacgtttgaggccttatcgtttaaaggctaacggaaatttctctaaag

SEQ ID NO: 31 - RNA, 373 nt, Varroa destructor; identical to SEQ ID NO: 23

SEQ ID NO: 32 - DNA, 693 bp, Varroa destructor
cgcctctatacagtgaaaaagtcggataaggttatgttactcagtaacttaaccttatcttggataacgttatttgacacgtaaacgaaaagtaataacaaagttttgtattatggctcgttattttcgagaggaagatatagatgaattcagggaatgtttttatctatttgcaaggaatggtcaaatacgtactttggatgagcttacaatcattatgagatcattaggattaagtccaactattgcagaattaaataaatatttgaaagataaaggtggaaaaatgtcttttgccgatttcttggaagttatgcatctacaaactagagctgaagatttaccaaaagaagtgatagatgcttttcaagctgcagataaatttaggactggcactataccagctagacagttagcgcatatgttactccactggggtgaacaattaagtaacaaagaagtggagcaaattttcagagaggcaaatgtgtctccaaatggacaagtaaagtacgaagattttgttaaaatagcttgtgcacctgtacctgattactattaaaataaatatttttcatattttttaaagatatttatatactttttacacaatacacacgtatttaattaataaaaggataaaaatgatcataaaagaaaaagaatttattcttccagcaacttatcttcgac

SEQ ID NO: 33 - RNA, 315 nt, Varroa destructor
augcuuuucaagcugcagauaaauuuaggacuggcacuauaccagcuagacaguuagcgcauauguuacuccacuggggugaacaauuaaguaacaaagaaguggagcaaauuuucagagaggcaaaugugucuccaaauggacaaguaaaguacgaagauuuuguuaaaauagcuugugcaccuguaccugauuacuauuaaaauaaauauuuuucauauuuuuuaaagauauuuauauacuuuuuacacaauacacacguauuuaauuaauaaaaggauaaaaaugaucauaaaagaaaaagaauuuauucuu

SEQ ID NO: 34 - DNA, 612 bp, Varroa destructor
cgtttttttaatttcaaagactcctgattttcttttcttttcctttcctacaaaccaaacacaagctagaaagaggttcgatttttgcaggaagaagaaggaacaatggctgatcagctcaccgatgaccagatctctgagtttaaggaagccttcagcctcttcgataaggatggagatggttgtatcaccaccaaggagcttggaactgtgatgaggtctcttggccagaaccccactgaggcagagctccaggacatgatcaacgaggtggatgctgatggcaatggaacaattgactttcctgagttcttaaacctcatggccaggaagatgaaggatactgattctgaggaggagctcaaggaagctttccgcgtgtttgacaaggaccagaatggcttcatttctgcggctgagctccgccatgttatgacgaatcttggtgagaagctcacagacgaggaagttgatgagatgatccgtgaggctgatgtagatggtgacggccagattaactacgaggagtttgtcaaagtcatgatggccaagtgaggatcattaaccaaaccttaaaatttcgaaagcataaacatttaaaaaaaaaaaaaa

SEQ ID NO: 35 - RNA, 371 nt, Varroa destructor
cagaucucugaguuuaaggaagccuucagccucuucgauaaggauggagaugguuguaucaccaccaaggagcuuggaacugugaugaggucucuuggccagaaccccacugaggcagagcuccaggacaugaucaacgagguggaugcugauggcaauggaacaauugacuuuccugaguucuuaaaccucauggccaggaagaugaaggauacugauucugaggaggagcucaaggaagcuuuccgcguguuugacaaggaccagaauggcuucauuucugcggcugagcuccgccauguuaugacgaaucuuggugagaagcucacagacgaggaaguugaugagaugauccgugaggcugauguaga

SEQ ID NO: 36 - DNA, 659 bp, Ixodes scapularis
acaccgcgctcgacgagaactcgcgcaaggagcgcgtgctaacgccgatagctctcgtacaaaagaaaactaaagacttgacacgctcaataccgatctttcacattttcagcaaaatttgagcattccgaatatggacctgactccggaagagatcgcggacatcaagggagcgtttctgctgtttgaccgcaacggcgacggaaccatctccacgactgagctagagatggtcctccgcgccatgggcgaacggcccagtccttcccagctggcccgtatagtgcggcaaattgacagcgaccgcaatggaagcatcgacttccaagagtttctctttttcatggccggcaggatttcccacaaaggcctctccaaaagcgcagtcctcaaggccttccaactcttcgaccgcgatggcaatggatacatcaccagggaggaactcgtccacattttcacgcacgttgggcagagcatgagccaagaagacgccgaaaagataatccgcgaagtggatgtggacaaggacggaaagatccattacactgaattggtcaacaaggtgctgcccaccaagaagcaaaaagaagaaaccaaaacctagaaggtcgtcgcttggcacggtctttattattaaacaagtgctttatcgcttg

SEQ ID NO: 37 - RNA, 374 nt, Ixodes scapularis
agaucgcggacaucaagggagcguuucugcuguuugaccgcaacggcgacggaaccaucuccacgacugagcuagagaugguccuccgcgccaugggcgaacggcccaguccuucccagcuggcccguauagugcggcaaauugacagcgaccgcaauggaagcaucgacuuccaagaguuucucuuuuucauggccggcaggauuucccacaaaggccucuccaaaagcgcaguccucaaggccuuccaacucuucgaccgcgauggcaauggauacaucaccagggaggaacucguccacauuuucacgcacguugggcagagcaugagccaagaagacgccgaaaagauaauccgcgaaguggauguggac

SEQ ID NO: 38 - DNA, 549 bp, Ixodes scapularis
gattcgtccacttattttgtccctattcttcgtccgcagtcgtcctcgaggaaaagtgcgtcaggtgcgggctacaagcggaaactgagcggaaagccagaaccgagcgaggagcagaagaatgacatgaaggaagcgttcagtctcttcgatcccagtggcacgggcttcatggagtctaaagatatgaagtttgcaatgagagcactgggttttgaaccaaaaaaggaggaagtgaaaaaactgatagcagagattgacaagcaggggactggaaaaattcccttggaggagttcatgagcgtcatgtccacgaggctggctgagaaagacataaatgaggagattatgaaggcgtttcagctgtttgatgaggatggcactgggaagatttcttttaagaacctcaagaatgtggccaaggaactgtcggagaacctcacagatgaggagcttcaggaaatgatcaatgaagctgacagggatggagatggcgaagtgaaccaagaggagttccttaggataatgaagaagacctgcctctactga

SEQ ID NO: 39 - RNA, 373 nt, Ixodes scapularis
ugaaggaagcguucagucucuucgaucccaguggcacgggcuucauggagucuaaagauaugaaguuugcaaugagagcacuggguuuugaaccaaaaaaggaggaagugaaaaaacugauagcagagauugacaagcaggggacuggaaaaauucccuuggaggaguucaugagcgucauguccacgaggcuggcugagaaagacauaaaugaggagauuaugaaggcguuucagcuguuugaugaggauggcacugggaagauuucuuuuaagaaccucaagaauguggccaaggaacugucggagaaccucacagaugaggagcuucaggaaaugaucaaugaagcugacagggauggagauggcgaagu

SEQ ID NO: 40 - DNA, 234 bp, Ixodes scapularis
atggccaagaacgtccgcgccctggacaccgaggaggagattttggaggccttcaaagtcttcgaccgcaacggcgacggcttcgtgagcacagccgagctccgtcacgtgatgaccacgttaggcgagaagttgacgcacgaagaagtggacgagatgatccgcgaggccgaccgcgacggcgacggacagatcaactacgacgagttcgtggccatgatgacttccaagtga

SEQ ID NO: 41 - DNA, 213 bp, Ixodes scapularis
cctggaaccgaggaggagattctggaggccttcaaagtcttcgaccgcaacggcgacggcttcgtgagcacggccgagctccgtcacgtgatgaccacgctaggcgagaagttgacgcacgaagaagtggacgagatgatccgcgaggccgaccgtgacggcgacggacagatcaactacgacgagttcgtggccatgatgacctccaagtga

SEQ ID NO: 42 - RNA, 200 nt, Ixodes scapularis
gaggaggagauucuggaggccuucaaagucuucgaccgcaacggcgacggcuucgugagcacggccgagcuccgucacgugaugaccacgcuaggcgagaaguugacgcacgaagaaguggacgagaugauccgcgaggccgaccgugacggcgacggacagaucaacuacgacgaguucguggccaugaugaccuccaa

SEQ ID NO: 43 - DNA, 450 bp, Aedes aegypti
atgtccgcccatagtctaacagaggaacaagggcgccagttccgtcagatgttcgagatgttcgacaaaaatggcgacggttcgatcagcacatcggaactgggatcggtcattcgggccttgggtatgaatccctccattgcggaaatcgagcaaatgatccacgaggtcgatttggacggaagtgggtcgattgagttgaacgaatttctcatactgatggcacgtaagtcacgggagggttccacacaggaagagctacgggatgcgttcaaaatttttgacaaggatggagatggatttctcacggttgacgagttgtcggctgttatgaagaactttggcgagagattgaccgatgacgaactagcagatctgctggaggaagccgacatcgatggagacggaaagatcaactatgaagaatttgtcatcatgttgagcaagtga

SEQ ID NO: 44 - RNA, 300 nt, Aedes aegypti
acagaggaacaagggcgccaguuccgucagauguucgagauguucgacaaaaauggcgacgguucgaucagcacaucggaacugggaucggucauucgggccuuggguaugaaucccuccauugcggaaaucgagcaaaugauccacgaggucgauuuggacggaagugggucgauugaguugaacgaauuucucauacugauggcacguaagucacgggaggguuccacacaggaagagcuacgggaugcguucaaaauuuuugacaaggauggagauggauuucucacgguugacgag

SEQ ID NO: 45 - DNA, 465 bp, Aedes aegypti
atgtccgcccaaaccccgccagacaagctttcccaggatcaaatcgaagaactgcgggaagctttctccctgttcgacaccaacggcgacggaaccataacctgttcagaacttggcacagtccttcgatcccttggcaaaaatgtatccgacgcggaagtggaagaactgctcaaagaagtcaacgtcgaccacgaaggaatgatccactttccggacttcgtggcaatgatgtccatccgattgcgggacttcaatagcgaggaggaactcaaggaagccttccggatcttcgaccgcaacggagatgggctgatttcggcggacgaattgcgagcggctctccaatctttcggggaacagctggccgaggaggaaatcgaagaactgctccgggaggcggatgtcaactgcgacggacaaatagactacgaggagtttgttaaaatgatcacgctgaaataa

SEQ ID NO: 46 - RNA, 300 nt, Aedes aegypti
caaaucgaagaacugcgggaagcuuucucccuguucgacaccaacggcgacggaaccauaaccuguucagaacuuggcacaguccuucgaucccuuggcaaaaauguauccgacgcggaaguggaagaacugcucaaagaagucaacgucgaccacgaaggaaugauccacuuuccggacuucguggcaaugauguccauccgauugcgggacuucaauagcgaggaggaacucaaggaagccuuccggaucuucgaccgcaacggagaugggcugauuucggcggacgaauugcgagcg

SEQ ID NO: 47 - DNA, 1150 bp, Aedes aegypti
tcgtcaaggatatccggcaactgattatgacccggcaaaccaacgatcccaacggccagcaacaggaacagaacgaaccagaatccagtcagaacacccagagcgaccaaagcaacaaccagcccacgcagcgattgggaggaaccacctcggacttcagtgtcagctccgcggccactaatcgaagtatgccccgccaccaggaggacaatcccaatcaaccggccagcgactgttccagcctcgagggaaatgtattcgtcgaaggcggatccggcaccggagcgcacccgaaaacacgccgctcgcaaacttccgattcgatcacctccagcaacttcaactacagtctcaaccggaggttcatatcgaagaaccagatgaaggagtttcgagaagcgttccggctgttcgacaaggataatgacggctcaatcaccaaggaagaactgggaactgtcatgaggtcgttgggacaatttgctcgcgtggaagaattacaagagatgttactggagattgatgttgatggcgatggaaacgtaagtttcgaagagtttgtcgacatcatgtccaacatgacggataccgtggcggaaacatcggccgaccaggaggaacgtgagctacgtgatgccttccgtgtcttcgacaagcacaatcgaggttacattacggcatcagatctacgggcggttcttcaatgtctgggcgaagatttggatgaagaagaaattgaagacatgatcaaagaagtggacgtggatggagacggacggatcgatttctacgaattcgtacatgctcttggagaaccggaagattcccaagaaaacgacgacgaagacgaggcagtgtccccccattcgctgtcctgtgacgtgcatgtctaagaaccgccaggagaaaaatagctaacgccaacgaatcgcattcctaacaaaatgtcgaacaatctagagacattgaccagattttttttaaatatttaacacacaaaaaaacttcgcttaacgccattgtacttctccatacgcttgataacagattccagaacacctaatgaatttatcaatctatacataataactattcatctctaatcacgaaaaaagtttaaataaacatatcaaattgagcaaccaataag

SEQ ID NO: 48 - RNA, 300 nt, Aedes aegypti
gaguuucgagaagcguuccggcuguucgacaaggauaaugacggcucaaucaccaaggaagaacugggaacugucaugaggucguugggacaauuugcucgcguggaagaauuacaagagauguuacuggagauugauguugauggcgauggaaacguaaguuucgaagaguuugucgacaucauguccaacaugacggauaccguggcggaaacaucggccgaccaggaggaacgugagcuacgugaugccuuccgugucuucgacaagcacaaucgagguuacauuacggcaucagau

SEQ ID NO: 49 - DNA, 450 bp, Culex quinquefasciatus
atgtcggcccactcgctcaccgacgaacagcagcgccagtaccggcaaatgttcgaaacgttcgacaaggatggcaacggttccatcacgacgacggaactgggaacgctagtgcgagcgctaggtcttaatccttcgatcgccgagatcgagcagatgatccacgaggtcgacctggacggaagcgggacgatcgagctgaacgagttttacgtgctgatggcccggaagcatcgggaagcctcgtcggaggacgagctgaggcaggctttcaaggtgtttgacaagaacgaggatgggttcttgacggtggaggaactgtcgatggtgatgaagaactttggtgagcggttgagcgatgaagagttggcggatttgttggaggaggcggatgttgacaaggacggtcggattaattacgaggaatttgtgaccatgttgaccaagtag

SEQ ID NO: 50 - RNA, 300 nt, Culex quinquefasciatus
acagcagcgccaguaccggcaaauguucgaaacguucgacaaggauggcaacgguuccaucacgacgacggaacugggaacgcuagugcgagcgcuaggucuuaauccuucgaucgccgagaucgagcagaugauccacgaggucgaccuggacggaagcgggacgaucgagcugaacgaguuuuacgugcugauggcccggaagcaucgggaagccucgucggaggacgagcugaggcaggcuuucaagguguuugacaagaacgaggauggguucuugacgguggaggaacugucgau

SEQ ID NO: 51 - DNA, 477 bp, Culex quinquefasciatus
atgtcatcgtcttcccgccaccccaaacccaccgcggaccccctgaccaaggagcaaatcgaagaactgcgcgaagcgttcaccctgttcgacaccaacggcgacggaacgatttccggctcggaactgtccaccgtgctgcgggccctcggcaagaacgtctcggacgccgaagtcgaggaactgctgaaggaggtccgcaccgacgacgagggccgcatccggttcggggactttgtggccatgatgacggtccggttgaaggactttaacaacgaggaccagctgcaggaggcgtttcggatcttcgatcgggacgggaatgggcggatttcggcggaagagctacgggtcgcgttgaggtcgtttggggagcagttgaccgaagaggagctggaggagttgctgcgcgaggcggacgtcaacagtgacggccagattgactacggggagtttgtgcggatgataacgcagtga

SEQ ID NO: 52 - RNA, 300 nt, Culex quinquefasciatus
gcgaagcguucacccuguucgacaccaacggcgacggaacgauuuccggcucggaacuguccaccgugcugcgggcccucggcaagaacgucucggacgccgaagucgaggaacugcugaaggagguccgcaccgacgacgagggccgcauccgguucggggacuuuguggccaugaugacgguccgguugaaggacuuuaacaacgaggaccagcugcaggaggcguuucggaucuucgaucgggacgggaaugggcggauuucggcggaagagcuacgggucgcguugaggucguuug

SEQ ID NO: 53 - DNA, 927 bp, Culex quinquefasciatus
atgaccgattttctccagcttccccaatgcaatactcgacaaaccaacgacccaaacagcgccgagcagcaacaacagagcgaacccgaatcgaaccagagcagcacgcaccagagcagcagccacagctaccagcagccgtcgtcaacgcagcaccggttggccggatctccgtcgagcagtgccaacgcgagtcccgtgatcggccggaacatgccccgccaccagcaccaggacaccgcgcccagtgacgatgggacctcgagcagtctggacgggagtgtctttgccgccgacggaactccgaccgctccgggggcgttggccaggacgcgccgctcgcagacctcggaatcgatcacctccagcaacttcaactacagtttgaaccggaggttcatctccaagaaccagatgaaagagttccgggaggcgttccggctgtttgacaaggacaacgacgggtcgatcacgaaggaggagctgggcacggtgatgcgatcactggggcagtttgcccgtgtcgaggaactgcaggagatgctgctggagattgacgtcgatggtgatggcaacgtcagcttcgaggagtttgtcgacatcatgtccaacatgaccgacacggtggcggaggcatccgccgaccaggaggagcgcgaactccgggatgcgttccgcgtgtttgacaagcacaaccggggctacatcacggcgtctgatctgcgggcggttctgcagtgtctgggagaagatttggacgaggaagaaatcgaagacatgatcaaggaggtggacgtcgacggcgatggacggatcgacttttacgagtttgtgcacgccctcggagagccggaagattcacaggagaacgacgacgaggaggaccccctgtcacctccgtcactgtcgtgtgacgtaaacgcctaa

SEQ ID NO: 54 - RNA, 300 nt, Culex quinquefasciatus
gaguuccgggaggcguuccggcuguuugacaaggacaacgacgggucgaucacgaaggaggagcugggcacggugaugcgaucacuggggcaguuugcccgugucgaggaacugcaggagaugcugcuggagauugacgucgauggugauggcaacgucagcuucgaggaguuugucgacaucauguccaacaugaccgacacgguggcggaggcauccgccgaccaggaggagcgcgaacuccgggaugcguuccgcguguuugacaagcacaaccggggcuacaucacggcgucugau

SEQ ID NO: 55 - DNA, 333 bp, Culex quinquefasciatus
atggtcggtgtccaagctggccatttgatatctcaatcacggcggggcggctccgcgtgcgaaaacggggaaattttgattgatgacggcggcggcggggagcggcgggttttaaacctgttctacaaggggaataaaaatgccgatcaacttacagaggaacagatcgccgagttcaaagaagcgttctcgctgttcgacaaagacggtgacggcacgatcacgaccaaggagctgggcaccgtgatgcgatcgttaggccagaaccccacagaagcagagctgcaagacatgataaacgaggtcgatgcggacggactgcatccgctttaa

SEQ ID NO: 56 - RNA, 300 nt, Culex quinquefasciatus
gucgguguccaagcuggccauuugauaucucaaucacggcggggcggcuccgcgugcgaaaacggggaaauuuugauugaugacggcggcggcggggagcggcggguuuuaaaccuguucuacaaggggaauaaaaaugccgaucaacuuacagaggaacagaucgccgaguucaaagaagcguucucgcuguucgacaaagacggugacggcacgaucacgaccaaggagcugggcaccgugaugcgaucguuaggccagaaccccacagaagcagagcugcaagacaugauaaacgag

SEQ ID NO: 57 - DNA, 934 bp, Acyrthosiphon pisum
gctgtgcacgttttgtttacccgaaaaatgtgattcaaactttcagttttttaaatcttaactgcgttgtttaagaaaaaaaaaaccctaaatttattattgtttattaataataaatcaatcgatcgaataatcgtttgcgggtatacctaagtacgaagtaaaatatgagtgcacaaaatagtgataatgaccgttataaaaaggaatattcgagaataaggaaactgacgagtagatatgacatacggactcaatcaaatgaatttggtttgtcggaagatcaagttgcggaattcaaagaagcatttatgttgttcgataaagaccatgatggacggattactgaggcagaactaggagtggtcatgagatctttgggtcaaaggcctactgaaactgatttgcgaggtatggttaaagaagtggataaagatggcaatggtagtattgagtttgatgaattcctgctaatgatggctagaaaactaaaagcagcagatggcgaggaagaaatgcaccaagcttttaaagtatttgacaaaaatggcgatggattcataacatttgatgaactcaaacgtgttatgtgcagtatcggagaaaggctcactgatgaagaaattgaggacatgataaaagaagcagatttaaatggtgataaaaaaattgattataaagaatttattacaataataagttctaagaaataaaacgaattacggacttggatgtaccctcatatggcattcgttcctcatctgcatctgtgtcattggctgctaagactttacttaataataaaccttgatcttctctactagaataaaatagctctggatcctaaagtaaaatatacagtataattttaaaatagtcgtatacaaatttttttttaaatattgagtgtacctcatccattccagcaagtttc

SEQ ID NO: 58 - RNA, 372 nt, Acyrthosiphon pisum
ucaaguugcggaauucaaagaagcauuuauguuguucgauaaagaccaugauggacggauuacugaggcagaacuaggaguggucaugagaucuuugggucaaaggccuacugaaacugauuugcgagguaugguuaaagaaguggauaaagauggcaaugguaguauugaguuugaugaauuccugcuaaugauggcuagaaaacuaaaagcagcagauggcgaggaagaaaugcaccaagcuuuuaaaguauuugacaaaaauggcgauggauucauaacauuugaugaacucaaacguguuaugugcaguaucggagaaaggcucacugaugaagaaauugaggacaugauaaaagaagcagauuuaaa

SEQ ID NO: 59 - DNA, 2509 bp, Acyrthosiphon pisum
gatttttcgtttaaataacccccccgggtttcggataaactcggtgtgcgtgtggacgccgccgccgccgcgtgagcgttatttcgctcgctgtgattacgaacgctcgtgcagtcgtcgtcatgcagcatctccgagacccggcgaaagaccatcagagtacgtgaacactgcacatcacactccatcgcgatatacttatctgtaggacgacaccctttaccgaggacacaatgatatacacgttataatactatcgtacatcgtatatattgtattcttatcatctaatattatattatcacaatcgttatattgtattatagaattattgtatatcgttttaatttgacacgatacgacatttggtgttgagaatcgcgcagagagagaaagagagagagaaaaagagagaatagatattttgatgtaaataattattacaatataatattgtatttgaaaatagaaacagataattggtcgttgaggcagttctcacctttttaagatatacatattatattatatataaacagtattttgttttactcctttgagtgaacatttcgtttaactataccacaatttattaatattatataatatctatcatggacggtaaaatatcatcggtattcgaaaaatacttttcaccttcaccgctggtgaaccaaataaggaattttgtcaatcggcaaatagacgagcaaacgccacaaaacgtaagcacacaaccaaccgctgtagcgaaacttcacagtaataatgtagtgaacggcaccactccgaaacccatcacaagcaacgaaaaaccaacggaagtccaagtacatccacaacccactcagcctgccgatagaaacttagtgcacgttactaaagcacagatgaaagaatttcaagaagcatttaggttatttgataaagacggtgacggcagcatcactaaagaggaattgggtcgagttatgcggagtcttggacagtttgctagagaagaagaattggagacaatgttacaagaagtcgacatcgatggcgatggagcgttcagttttcaagagtttgtagaaattgtgtacaatatgggtggtacagcagaaaagacggcggaccaagaggaaaaagagctccgagacgcatttagggtatttgacaaacataaccgaggatatataagtgcgtcggacttgagagctgtccttcaatgtttgggtgaagatttgtcagaagaagaaatcgaggatatgatcaaggaagtagacgtggacggagatggaagaatcgatttttacgaatttgtgaatgcccttggagaaccaggagatgattatgatgaaaacgacgaagatgaagaagatatttatccccaattggacattcaaacataacttataaacaattacacgttttagtatgatgcgataacaagttcagttaaaattgaattatcaaaaatgataacaatattttttgtaaacttaggttaaaatgttaaaaacttacccattttgtaatttctatcaggaataaacacaccaatatctgttttttttttgccaactaatgatctctaataagtaaaacatattttactttaatatcaatgtactactgtagtattgttaagtaatttatgtcattttcaatgtttaatgtataaattaatcatttaatggtacaatcagtaattcaccttaagacccaattatttattaaaaacatattatatcattaatttacttaatgtatacattttagtcaaaaaacattcagttatatgttataagtcgttataactatttatttaagaaactataaaaaattattatttattataatagtttacgtatctatttacttccatggaaggtatttataaatagaaaatgttaaggtaacttaattaaaacaataattatgaacaagtatttttactttaaaaaaattacataattatattgtcagtattctttcaaatacaattaattcaaatttgtgaaattgtccattcctcctttatgctttgtgaactaaatttaaatacattaagaaccagagtacaattaaaggaaatagtcagctgcgtgtttttttgttggcattcctcggttttcttgtggtgctgcctcaaatattgtaaaatctctttgaagtgtttcactgagttccaatattgccgcaacgttaccacatctattatttacaattagtattaacaattaaataacagcattaataaataaatagtataatgtaatttttagagtagtatttaccgataacaatagttgggtgctgaccaaacagtaagcacggtttcatcaaaatgccatttatatccttccatgactagttgatgagctcgacaaataatatctatatcatttgtagtattaaactgggagacaacatcagaaccaaataggtatccagcaccccgaggactcacaccccatccctgagtatctaaaataattgtgtatgttaaaaatctatttttttt

SEQ ID NO: 60 - RNA, 294 nt, Acyrthosiphon pisum
acagaugaaagaauuucaagaagcauuuagguuauuugauaaagacggugacggcagcaucacuaaagaggaauugggucgaguuaugcggagucuuggacaguuugcuagagaagaagaauuggagacaauguuacaagaagucgacaucgauggcgauggagcguucaguuuucaagaguuuguagaaauuguguacaauaugggugguacagcagaaaagacggcggaccaagaggaaaaagagcuccgagacgcauuuaggguauuugacaaacauaaccgaggauauau

SEQ ID NO: 61 - DNA, 477 bp, Pediculus humanus
atggccgacgaaacgacgacggaattaccggaggaaaatctttcggttgaaaaaatcgcagaattccgcgaagctttcaaccttttcgacaaagatggcgacggtaacataacgaccaaagaattgggtacttgcatgaggtctctcgggcagaatccgacggaagcggaaatcgcggagctgatttgcgaagtagacgtagagggaacaggtttaatcgatttcacatcgttcgttttgataatggctaaaaagataaaagacgtcgacaacgaggaagaactcagagaagcttttagaatattcgataaggaaggtaacggattcataaccgcatccgagctcaggcacataatgatgaacttgggtgaaaaattaacggaagaagaatgcgacgaaatgattagggaagcggatgtcatgggtgacggaaatatcaattacgaagaattcgtcaccatgatgatgtcaaagtga

SEQ ID NO: 62 - RNA, 379 nt, Pediculus humanus
aaaaaucgcagaauuccgcgaagcuuucaaccuuuucgacaaagauggcgacgguaacauaacgaccaaagaauuggguacuugcaugaggucucucgggcagaauccgacggaagcggaaaucgcggagcugauuugcgaaguagacguagagggaacagguuuaaucgauuucacaucguucguuuugauaauggcuaaaaagauaaaagacgucgacaacgaggaagaacucagagaagcuuuuagaauauucgauaaggaagguaacggauucauaaccgcauccgagcucaggcacauaaugaugaacuugggugaaaaauuaacggaagaagaaugcgacgaaaugauuagggaagcggaugucaugggugac

SEQ ID NO: 63 - DNA, 537 bp, Pediculus humanus
atggatgctaggaatgaagtttacaacaccgaatataatcgtttaagaaaattgacgtgtagaacggaaattaaattatcttgctctgaatatggtcttacggaggaacaagtcgctgaatttaaagaagcttttatgctttttgacaaagatgaagatggacaaataacaatggccgaattaggagtcgttatgagatctttgggacaacgtccgacagaaacggaattaagagacatggttaaagaggttgatcaagatggaaatggtacaatcgaattcaatgaatttttacaaatgatggcaaaaaaaatgaaaggagctgatggtgaagaagaacttcgagaagcattcagggtgtttgataaaaataacgatggactcatttcatccattgaacttcgacatgtcatgacaaatttaggtgagaaactttcagacgaagaagttgatgatatgataaaagaagcagatttagatggagatggtatggttaactacaatgaatttgtaacgatattaacatcaaaaaattaa

SEQ ID NO: 64 - RNA, 417 nt, Pediculus humanus
acaagucgcugaauuuaaagaagcuuuuaugcuuuuugacaaagaugaagauggacaaauaacaauggccgaauuaggagucguuaugagaucuuugggacaacguccgacagaaacggaauuaagagacaugguuaaagagguugaucaagauggaaaugguacaaucgaauucaaugaauuuuuacaaaugauggcaaaaaaaaugaaaggagcugauggugaagaagaacuucgagaagcauucaggguguuugauaaaaauaacgauggacucauuucauccauugaacuucgacaugucaugacaaauuuaggugagaaacuuucagacgaagaaguugaugauaugauaaaagaagcagauuuagauggagaugguaugguuaacuacaaugaauuuguaacgauauuaac

SEQ ID NO: 65 - DNA, 648 bp, Pediculus humanus
atgactacgaaacataatatatctggaagaatacgggacgaaccagggggacaaagggaaaaaaatggaaatgtaaccggtcgaacaataacatatccaacaacagggaacaaaagaaatattgatacaatgacgaaaaataacatatcaaaatcgcaaatgaaggaatttcgagaagcttttcgactttttgacaaagatggtgatggtagtataactcaagaagaacttggaagagttatgagatctttaggacaatttgccagagaagaagaactacaagaaatgcttaaggaagttgatatagatggagatggaaattttagctttgaagaatttgttgaaatcgtatcaaatatgggaggtgcagcaactgaaaaaacagctgatgaagaagagaaagaacttagagatgcttttagagtatttgataaacataatcgaggttttataagtgcttctgatcttcgagctgttttgcaatgtctgggtgaagaattatcagaagaagaaaaaatgataagagaagttgatgtggatggagatggtagaattgattttttcgaatttgttcgagctttgggtacacactacaggcaaaatttctttttcaggtttctatccatttatattattagcacagtttga

SEQ ID NO: 66 - RNA, 449 nt, Pediculus humanus
aucgcaaaugaaggaauuucgagaagcuuuucgacuuuuugacaaagauggugaugguaguauaacucaagaagaacuuggaagaguuaugagaucuuuaggacaauuugccagagaagaagaacuacaagaaaugcuuaaggaaguugauauagauggagauggaaauuuuagcuuugaagaauuuguugaaaucguaucaaauaugggaggugcagcaacugaaaaaacagcugaugaagaagagaaagaacuuagagaugcuuuuagaguauuugauaaacauaaucgagguuuuauaagugcuucugaucuucgagcuguuuugcaaugucugggugaagaauuaucagaagaagaaaaaaugauaagagaaguugauguggauggagaugguagaauugauuuuuucgaauuuguucgagcuuuggguacacacuacaggcaaa

SEQ ID NO: 67 - DNA, 648 bp, Pediculus humanus
atgatgaaaaacaaaactgacagcagtctcggagctgagcattcagatttgaaacattcgacgagtgaaaccgaagaactccaatcctcggaactcgaagtgataaaagatgaagagcctcaaatagatctgagacagtttctgacgaaagaacaagtgcaagaattcaaaagaattttccaggcttacgatgtcaacaacgaagataaaatcccggtcaaagccatcggaatcattttgagaaacatgggattgaatccgtccaaggcgattctcaagagaatgacaaaggaaatcgatccggataaaaacggttacgtggatttcgaaatgtttttacatcccatggcacgaatgatacacgaagtcccggaaaatcacgaggacataatcgcagcattcaaagttttcgacgaagacgacgaaggtttcgtatccgttaaagctttgaccgaatacctcacgaacctgggcgaagatttggaagatttcgaaattgataatttgattaaaatggcggatcccaaaggcacgggccgagtctactacgaaggattcgtcgagaaaattttcggaatcgtaagaaacgggaaaaaaaagaaaaatctcaaagggaaaaagggaaaaaaacgaaaaaaaaatgaatga

SEQ ID NO: 68 - RNA, 451 nt, Pediculus humanus
ucaaauagaucugagacaguuucugacgaaagaacaagugcaagaauucaaaagaauuuuccaggcuuacgaugucaacaacgaagauaaaaucccggucaaagccaucggaaucauuuugagaaacaugggauugaauccguccaaggcgauucucaagagaaugacaaaggaaaucgauccggauaaaaacgguuacguggauuucgaaauguuuuuacaucccauggcacgaaugauacacgaagucccggaaaaucacgaggacauaaucgcagcauucaaaguuuucgacgaagacgacgaagguuucguauccguuaaagcuuugaccgaauaccucacgaaccugggcgaagauuuggaagauuucgaaauugauaauuugauuaaaauggcggaucccaaaggcacgggccgagucuacuacgaaggauucgucgagaaaauu

SEQ ID NO: 69 - RNA, 1546 nt, Varroa destructor
guuuagcccauuuucgcgcugugucugucggcgacugcggaaguacugagcuagcugagucguggugcuuagaaggcaguggcagugaguggcaucagcgguaauaagugagggacaacagccggagagucgugucgguugguaggucgguucguugccgauuaaugccccacaugugaguuacgugcggugcuuguuccgcugugcauuggacguuacauacagagagucagguguaguuuauuuuagacgaaaaacuaccagcacuaccugauacagcgacccaacguagagagggaaagagaaagagcuguuguuucgcuagguuaguucugaacaauuggauugauucgcaaauguacgcuuguacggcuaacgguugaacggacugugcaaacugcggauagugcgugaacuagcagacaacauauccaauaacuaacuacacgguuauuauugauacaaacaccuaguucagacagacaauuucgguuugcuuuguuggcacuauaaggaguaagugauauuguuuuuuguuuaucagucggccuaguauugucggugcacuuacggauaacaggagaggcaguacaaaggcaacucgauucacuaucguucacgggcgcuaauacagcgaaauauuaauaggcaaagcaagcaagccagccggccaagcccaaaccccgggcgaaacgcagauaccaacagcgcugaagugcguggcaaacgacaacgggacaguagggcauaagcuagacagcauauagcuuuucuaaccauggcugaucagcuaacugaggaacagaucgccgaguucaaagaggcguuuagccuguuugacaaggacggagauggcacgaucacgacaaaggagcucgguacgguaaugcgaucucucggccagaaccccacugaggcugaacugcaggacaugaucaacgaggucgacgccgacggcuccggaacgauagauuucccugaguuccucacaaugauggcaagaaagaugaaggacaccgacucggaggaggagauccgagaggcguuccgcguauucgacaaggauggcaacgguuucauuucggcggccgagcucaggcacguuaugaccaaccuuggcgagaagcuuacggacgaggagguagaugagaugauucgggaggcagauauugacggugauggucaggucaacuacgaggaguucgucaccaugaugacguccaaguaaauauaugauaauguuggcugucucguguaaugucgugagaaagaaagcgcgcgcgaaagaaagagagaaaggaauagaaaacuauaaauagcuuguuguuaaagcaacgcaacaacaagcuguaagcaacaaacaauauuuacgaaguauacgauaaugaaagucgacagggaagcaagcacggauauauaugaaaacuaagcgaaaugacgucgucaucaucaccagcagcagcagcagcagcagcagcagcagcagcagcaccaccaccaccaccaucacgaccaccaccaccaccaccaccaucacgaccaccac

SEQ ID NO: 70 - RNA, 1136 nt, Varroa destructor
guucggcucggggacuagcugaucggucgguguguauuguuggcuauuggcaaagaccguuguugagugggcucgcugcacugagcguuuaaaucuggugaaaucguuggcaauggcggaucagcugaccgaggagcaaaucgccgaauucaaggaggcuuucagccuguucgauaaagacggugauggcacaauuacgaccaaggaacuagggaccgucaugcggucccucggccagaacccuacugaggcugagcuucaagacaugaucaacgaggucgacgcugacgguaacggcacuauugacuuuccagaguuucucacgaugauggcgcguaaaaugaaggacaccgacuccgaggaggagauccgggaagcuuuuaggguuuuugauaaagacggaaauggcuucauuucggcugcagagcugaggcacguaaugaccaaccuuggcgaaaagcucacggacgaggaaguggacgagaugauccgcgaggcggauaucgacggcgacggacaggucaacuacgaggaguucgucacgaugaugacaucaaaaugaagggcucacuauugcgcgggaaaagcagcccaacaaagaaaccuagagugcgaaagcgagaacguuaaacacgaugauaugcuaaugauaauacauacgacuagaggacagaaagacagacagacagacugagcagacgaacgggcaaguugaagaaaagccgaguugaacuggcuaaccguuggguacucauucauauucgauaguuacagacaacaacaugaaaaacgacagcaacaauccgcaacaaacacacggagauugcacacaaugaggguaaacugaacauggugcagcggaaguuggauggcagcgguacacagugcugcuacugcugcugcugcaaaugcuaacacucaauaaugauaauaauaauuauaauuauagaaauaugauuauguuguccaaaagagaaacaaacaacacaaacaaagcuauuaaaaaucugaauaaaagcuaagaagaaaucaaguagcagucgacauggggaguggcaaacgauaagaguccacagaaaacugaagcggccgaaagaaaacacgaggcaaaaggcaauguauucauuaagacgagg

SEQ ID NO: 71 - RNA, 150 nt, Artificial Sequence
  Synthetic Sequence
guuuagcccauuuucgcgcugugucugucggcgacugcggaaguacugagcuagcugagucguggugcuuagaaggcaguggcagugaguggcaucagcgguaauaagugagggacaacagccggagagucgugucgguugguaggucgg

SEQ ID NO: 72 - RNA, 150 nt, Artificial Sequence
  Synthetic Sequence
uucguugccgauuaaugccccacaugugaguuacgugcggugcuuguuccgcugugcauuggacguuacauacagagagucagguguaguuuauuuuagacgaaaaacuaccagcacuaccugauacagcgacccaacguagagagggaa

SEQ ID NO: 73 - RNA, 150 nt, Artificial Sequence
  synthetic sequence
agagaaagagcuguuguuucgcuagguuaguucugaacaauuggauugauucgcaaauguacgcuuguacggcuaacgguugaacggacugugcaaacugcggauagugcgugaacuagcagacaacauauccaauaacuaacuacacgg

SEQ ID NO: 74 - RNA, 150 nt, Artificial Sequence
  synthetic sequence
uuauuauugauacaaacaccuaguucagacagacaauuucgguuugcuuuguuggcacuauaaggaguaagugauauuguuuuuuguuuaucagucggccuaguauugucggugcacuuacggauaacaggagaggcaguacaaaggcaa

SEQ ID NO: 75 - RNA, 150 nt, Artificial Sequence
  synthetic sequence
cucgauucacuaucguucacgggcgcuaauacagcgaaauauuaauaggcaaagcaagcaagccagccggccaagcccaaaccccgggcgaaacgcagauaccaacagcgcugaagugcguggcaaacgacaacgggacaguagggcaua

SEQ ID NO: 76 - RNA, 150 nt, Artificial Sequence
  synthetic sequence
agcuagacagcauauagcuuuucuaaccauggcugaucagcuaacugaggaacagaucgccgaguucaaagaggcguuuagccuguuugacaaggacggagauggcacgaucacgacaaaggagcucgguacgguaaugcgaucucucgg

SEQ ID NO: 77 - RNA, 150 nt, Artificial Sequence
  synthetic sequence
ccagaaccccacugaggcugaacugcaggacaugaucaacgaggucgacgccgacggcuccggaacgauagauuucccugaguuccucacaaugauggcaagaaagaugaaggacaccgacucggaggaggagauccgagaggcguuccg

SEQ ID NO: 78 - RNA, 150 nt, Artificial Sequence
  synthetic sequence
cguauucgacaaggauggcaacgguuucauuucggcggccgagcucaggcacguuaugaccaaccuuggcgagaagcuuacggacgaggagguagaugagaugauucgggaggcagauauugacggugauggucaggucaacuacgagga

SEQ ID NO: 79 - RNA, 150 nt, Artificial Sequence
  synthetic sequence
guucgucaccaugaugacguccaaguaaauauaugauaauguuggcugucucguguaaugucgugagaaagaaagcgcgcgcgaaagaaagagagaaaggaauagaaaacuauaaauagcuuguuguuaaagcaacgcaacaacaagcug

SEQ ID NO: 80 - RNA, 150 nt, Artificial Sequence
  synthetic sequence
uaagcaacaaacaauauuuacgaaguauacgauaaugaaagucgacagggaagcaagcacggauauauaugaaaacuaagcgaaaugacgucgucaucaucaccagcagcagcagcagcagcagcagcagcagcagcagcaccaccacca

SEQ ID NO: 81 - RNA, 150 nt, Artificial Sequence
  synthetic sequence
guucggcucggggacuagcugaucggucgguguguauuguuggcuauuggcaaagaccguuguugagugggcucgcugcacugagcguuuaaaucuggugaaaucguuggcaauggcggaucagcugaccgaggagcaaaucgccgaauu

SEQ ID NO: 82 - RNA, 150 nt, Artificial Sequence
  synthetic sequence
caaggaggcuuucagccuguucgauaaagacggugauggcacaauuacgaccaaggaacuagggaccgucaugcggucccucggccagaacccuacugaggcugagcuucaagacaugaucaacgaggucgacgcugacgguaacggcac

SEQ ID NO: 83 - RNA, 150 nt, Artificial Sequence
  synthetic sequence
uauugacuuuccagaguuucucacgaugauggcgcguaaaaugaaggacaccgacuccgaggaggagauccgggaagcuuuuaggguuuuugauaaagacggaaauggcuucauuucggcugcagagcugaggcacguaaugaccaaccu

SEQ ID NO: 84 - RNA, 150 nt, Artificial Sequence
  synthetic sequence
uggcgaaaagcucacggacgaggaaguggacgagaugauccgcgaggcggauaucgacggcgacggacaggucaacuacgaggaguucgucacgaugaugacaucaaaaugaagggcucacuauugcgcgggaaaagcagcccaacaaag

SEQ ID NO: 85 - RNA, 150 nt, Artificial Sequence
  synthetic sequence
aaaccuagagugcgaaagcgagaacguuaaacacgaugauaugcuaaugauaauacauacgacuagaggacagaaagacagacagacagacugagcagacgaacgggcaaguugaagaaaagccgaguugaacuggcuaaccguugggua

SEQ ID NO: 86 - RNA, 150 nt, Artificial Sequence
  synthetic sequence
cucauucauauucgauaguuacagacaacaacaugaaaaacgacagcaacaauccgcaacaaacacacggagauugcacacaaugaggguaaacugaacauggugcagcggaaguuggauggcagcgguacacagugcugcuacugcugc

SEQ ID NO: 87 - RNA, 150 nt, Artificial Sequence
  synthetic sequence
ugcugcaaaugcuaacacucaauaaugauaauaauaauuauaauuauagaaauaugauuauguuguccaaaagagaaacaaacaacacaaacaaagcuauuaaaaaucugaauaaaagcuaagaagaaaucaaguagcagucgacauggg

SEQ ID NO: 88 - RNA, 156 nt, Artificial Sequence
  synthetic sequence
ggcaacgguuucauuucggcggccgagcucaggcacguuaugaccaaccuuggcgagaagcuuacggacgaggagguagaugagaugauucgggaggcagauauugacggugauggucaggucaacuacgaggaguucgucaccaugaugacgucc

SEQ ID NO: 89 - RNA, 257 nt, Artificial Sequence
  synthetic sequence
ggcggaucagcugaccgaggagcaaaucgccgaauucaaggaggcuuucagccuguucgauaaagacggugauggcacaauuacgaccaaggaacuagggaccgucaugcggucccucggccagaacccuacugaggcugagcuucaagacaugaucaacgaggucgacgcugacgguaacggcacuauugacuuuccagaguuucucacgaugauggcgcguaaaaugaaggacaccgacuccgaggaggagaucc